European Patent Application EP 4 234 690 A1, published August 30, 2023. Title: RECOMBINANT KOD POLYMERASE. Applicant: BGI SHENZHEN. The sequence listing filed with the application follows.

SEQUENCE LISTING (6 sequences)

SEQ ID NO: 1 - protein, 774 aa, Artificial sequence
MILDTDYITEDGKPVIRIFKKENGEFKIEYDRTFEPYFYALLKDDSAIEEVKKITAERHGTVVTVKRVEKVQKKFLGRPVEVWKLYFTHPQDVPAIRDKIREHPAVIDIYEYDIPFAKRYLIDKGLVPMEGDEELKMLAFAIATLYHEGEEFAEGPILMISYADEEGARVITWKNVDLPYVDVVSTEREMIKRFLRVVKEKDPDVLITYNGDNFDFAYLKKRCEKLGINFALGRDGSEPKIQRMGDRFAVEVKGRIHFDLYPVIRRTINLPTYTLEAVYEAVFGQPKEKVYAEEITTAWETGENLERVARYSMEDAKVTYELGKEFLPMEAQLSRLIGQSLWDVSRSSTGNLVEWFLLRKAYERNELAPNKPDEKELARRRQTFEGGYIKEPERGLWENIVYLDFRSIAPSIIITHNVSPDTLNREGCKEYDVAPQVGHRFCKDFPGFIPSLLGDLLEERQKIKKKMKATIDPIERKLLDYRQREIKILANSYYGYYGYARARWYCKECAESVTAWGREYITMTIKEIEEKYGFKVIYSDTDGFFATIPGADAETVKKKAMEFLKYINAKLPGALELEYEGFYKRGFFHTKKKYAVIDEEGKITTRGLEIVRRDWSEIAKETQARVLEALLKDGDVEKAVRIVKEVTEKLSKYEVPPEKLVIHEQITRDLKDYKAKGPHMAVAKRLAARGVKIRPGTVISYIVLKGSGRIGDRAIPFDEFDPTKHKYDAEYYIENQVLPAVERILRAFGYRKEDLRYQKTRQVGLSAWLKPKGT

SEQ ID NO: 2 - DNA, 2325 bp, Artificial sequence
atgattctggacaccgattacatcaccgaagatggcaagccagttatccgcattttcaaaaaagagaatggtgaattcaagatcgaatatgatcgtaccttcgagccgtacttctatgctctgctgaaagacgatagcgcgattgaggaggtcaagaaaatcaccgcggagcgtcacggtacggttgttaccgtgaaacgcgtggagaaagtccagaagaaatttctgggtcgcccggttgaagtgtggaagctgtactttacgcatccgcaagatgttccggcgattcgcgataagattcgtgagcacccggcagtcattgacatctacgagtatgacattccgttcgccaagcgttatctgatcgataagggtctggtcccgatggagggtgacgaagaactgaagatgctggcgttcgccatcgccactctgtaccacgagggtgaagagtttgccgagggtccgatcttgatgatttcctacgcggacgaagagggcgcacgtgttatcacgtggaaaaatgttgatctgccgtatgttgacgtcgtaagcaccgagcgtgagatgatcaaacgttttctgcgcgttgttaaagaaaaagatcctgacgtgctgatcacctacaacggtgacaatttcgatttcgcgtacctgaagaaacgttgcgaaaaactgggtattaacttcgcgctgggtcgcgatggctctgaaccgaagatccagcgcatgggtgatcgttttgcggtcgaggtgaagggtcgcattcatttcgacctgtacccggtgattcgtcgtaccatcaacttgccgacttacaccctggaagccgtctatgaagctgtatttggtcaaccgaaagaaaaagtgtacgctgaggaaattacgacggcgtgggaaaccggtgagaacctggagcgcgttgcacgttattctatggaggacgcgaaagttacctacgaactgggtaaagagttcctgccgatggaggcccaactgtcccgtctgatcggccaaagcctgtgggacgttagccgcagcagcaccggtaacttagttgaatggttcttgctgcgtaaggcatacgaacgcaatgagctggcgccgaacaaaccggacgagaaagaattggcgcgtcgccgccagacctttgagggtggttatatcaaagaaccggagcgcggcttgtgggagaacatcgtctatttggattttcgtagcattgcaccgagcatcattatcacgcataatgtgagcccggatacgttgaatcgtgagggctgtaaggaatacgacgtggcgcctcaggttggccaccgtttctgcaaggactttccgggctttatcccgagcctgctgggtgatttgctggaggaacgtcagaaaatcaagaagaagatgaaagcaaccattgatccgatcgagcgcaaattactggactaccgtcaacgtgaaatcaagatcctggcgaattcgtattatggttactatggctacgcgcgtgcgcgctggtattgcaaagagtgtgccgagagcgtgaccgcttggggtcgtgagtacattaccatgacgatcaaagagattgaagagaaatacggctttaaggttatctatagcgacaccgacggtttctttgcaactatccctggcgcagacgcagaaaccgttaagaaaaaggcaatggagtttctgaagtatatcaacgcgaagttgccaggcgccctggaactggagtacgagggcttctacaagcgtggctttttccatacgaaaaagaaatacgctgttattgatgaagagggcaagatcacgacccgtggcctggaaattgtgcgccgtgattggagcgaaattgcaaaagaaacgcaagcgcgtgtgctggaagcgctgctgaaggacggcgacgtcgaaaaagctgtgcgtattgttaaagaggtcaccgagaagctgagcaaatacgaggtcccgccagagaaattggtgattcacgaacagattacgcgtgacctgaaagactataaggccaaaggtccgcatatggcagtggcgaagcgcctggcggctcgcggtgtgaagatccgtccgggtaccgtcattagctatatcgtgctgaagggcagcggtcgtatcggcgaccgtgcgattccgttcgacgaatttgatccgaccaaacacaaatatgatgcggaatactatattgagaaccaagtgctgccagccgttgagcgtattctgcgcgccttcggttaccgcaaggaagatctgcgttaccagaaaactcgtcaggtcggtctgtccgcatggctgaaaccgaagggcacctga

SEQ ID NO: 3 - DNA, 25 bp, Artificial sequence
ggtttttttatggggggagtttagg

SEQ ID NO: 4 - DNA, 25 bp, Artificial sequence
catctcatctgtaacatcattggca

SEQ ID NO: 5 - DNA, 37 bp, Artificial sequence
cgtgtatgcgtaataggatcccgactcactatggacg

SEQ ID NO: 6 - DNA, 37 bp, Artificial sequence
cgtgtatcgtccatagtgagtcgggatcctattacgc